European Patent Specification EP 3 717 650 B1, published June 18, 2025. Title: Transgenic Maize Event MON87429 and Methods of Use Thereof. Applicant: Monsanto Technology LLC. The sequence listing filed with the application follows.

SEQUENCE LISTING (13 sequences)

SEQ ID NO: 1 - DNA, 30 bp, Artificial Sequence
  Chimeric DNA molecule of maize genomic DNA and transgene DNA
ccactcttgtttggtttcatgtccgggaaa

SEQ ID NO: 2 - DNA, 30 bp, Artificial Sequence
  Chimeric DNA molecule of maize genomic DNA and transgene DNA
cggtgcacaaactatagcaagtgtggtcta

SEQ ID NO: 3 - DNA, 60 bp, Artificial Sequence
  Chimeric DNA molecule of maize genomic DNA and transgene DNA
acttgcaaaaatagaccactcttgtttggtttcatgtccgggaaatctacatggatcagc

SEQ ID NO: 4 - DNA, 60 bp, Artificial Sequence
  Chimeric DNA molecule of maize genomic DNA and transgene DNA
gcacaacaaacgcaccggtgcacaaactatagcaagtgtggtctatttttatatagcaag

SEQ ID NO: 5 - DNA, 100 bp, Artificial Sequence
  Chimeric DNA molecule of maize genomic DNA and transgene DNA
agatactcttgtttggttacacttgcaaaaatagaccactcttgtttggtttcatgtccgggaaatctacatggatcagcaatgagtatgatggtcaata

SEQ ID NO: 6 - DNA, 100 bp, Artificial Sequence
  Chimeric DNA molecule of maize genomic DNA and transgene DNA
atgacgtcccgcgatcgcccgcacaacaaacgcaccggtgcacaaactatagcaagtgtggtctatttttatatagcaagtgaggtcagataaaataata

SEQ ID NO: 7 - DNA, 1350 bp, Artificial Sequence
  Chimeric DNA molecule of maize genomic DNA and transgene DNA
atctacagggcgcgcagcggctgacacatgggacccacgggcaaaggcagcggcagactcgcgcgcgagagcacgcaagcaccgattgacgcgcgtgccccttttgtcggagaacgagggtgcgcgatcgtccgtgcatggttgagacggccaggcggggcccacccattggcgccatgccgcgcgagcagcagctggcccgcacaggtgcaaaggttgagtgggctagaagcgaagacctagtccaagcgacggtttcttccttttttctctttttttctttttcctttatattttcttgttttattttattttcatttttttattttcaaatctaaatttgaactcaagtgtgagattcatactttgaattaaatgctcacattcaaatatcagtaggaatagaatatttttaactatatgtttattttctctattttatacaatcttttccttttttcatttttaaacctcaatttgtaaattatatctaaattccaattttggtcattagtatactcctactaatatcattttattgttatgaaatgcacacacaataaactccaacttgatgaatagatatctatttattctaattaatttatttgtttggtagatgttcaaaatatgaaacacacacatattgttttctttctttttagaaaaatggtatttttattgtgggacaagaactaaaagtcacctcaaaattaaatactcatgtataatttgggatatctgaatttactatttttatttcttcatatatttaatttattattaattttttttcttattgggccttacacttatgagatcatagaggcatgtggatcagtggcatacaagttgaaattactgccaaaaatgtctgtcatacacaatccgtgtgtttggtttgtggaccagcagagcctggctactctaatccgtatgtagagaaccaagctcccacgagacagactcaatgtatccgagatactcttgtttggttacacttgcaaaaatagaccactcttgtttggtttcatgtccgggaaatctacatggatcagcaatgagtatgatggtcaatatggagaaaaagaaagagtaattaccaattttttttcaattcaaaaatgtagatgtccgcagcgttattataaaatgaaagtacattttgataaaacgacaaattacgatccgtcgtatttataggcgaaagcaataaacaaattattctaattcggaaatctttatttcgacgtgtctacattcacgtccaaatgggggcttagatgagaaacttcacgatttggcgcgactaactaagcactagcgtacgggacccagatatcgaattca

SEQ ID NO: 8 - DNA, 1069 bp, Artificial Sequence
  Chimeric DNA molecule of maize genomic DNA and transgene DNA
gatcgcccgcacaacaaacgcaccggtgcacaaactatagcaagtgtggtctatttttatatagcaagtgaggtcagataaaataataaataaaatcattaaattttatatagcaagtgtggtctatttttgcttgtaaactacagagaatatatatatgttaaatcggtagaacaattggctatttaaactaaaagatttaaaaaaaacaaagataaaaaatgtttttgaactgcgtgtctcgagagcagccagcatgcttccgacctgcatgagcagcgatgctcctggtgaccgcacgaacggaacctggcccgatggatgattttgcatcaacagcgcctgtatgcaacgatcatccaaccaaacatacttcgctttgaggatccacgcctacaacgtccgcgctcgtccatgcaaccaaacacacggaatgtgttccatgtgtcccaattgaaagaagtgtattcggttaacaacggaagtcataaccgagccagatatagagatagaaccagatctatcataccaagaacacccctccaagattctagactgcaaggaaagatccactcgtgcgaagacgaccaagatgtataagatccaatggagcaaccatacggaagaagaggctacgtgggagactgaggattatctatgcaaatactaccccgattgtctacctaaggaagtcagtacgtaaccatgccccagccccctgccctccgattccaaatatagaaaagatactcttaatgaaaactgaattaagaaatgaaattaagcgaagaaggacttccttctgaagttgcaaagaggatggcattcgaagagcagatttttctcgcgaaccttaaaaagctaaccaatactatgcaagcaagctataaccacctcctcactcctgggtgatctcgactcgaatctcggggcgagattcttttaaggggggagagctgtaacaccccaggtgttacttagggtttcccccttagtacctccatttgtgacctattatcacatgtggtttggtttaagaaaaaggcaccaaacttgaggggccaagccc

SEQ ID NO: 9 - DNA, 14008 bp, Artificial Sequence
  Transgene insert
ttcatgtccgggaaatctacatggatcagcaatgagtatgatggtcaatatggagaaaaagaaagagtaattaccaattttttttcaattcaaaaatgtagatgtccgcagcgttattataaaatgaaagtacattttgataaaacgacaaattacgatccgtcgtatttataggcgaaagcaataaacaaattattctaattcggaaatctttatttcgacgtgtctacattcacgtccaaatgggggcttagatgagaaacttcacgatttggcgcgactaactaagcactagcgtacgggacccagatatcgaattcaagctgaccgccaccggcaaacaaccacgaatttgtaatggtactaggcaaattctccgtttggcggtgtgtgccggccaattacacgtttttgcggtgtcctccgacaaaatttgccttttaaaaacaattttataagagaagctccggagataaaaggccgtcaatgttacaagagtgaagtcgtctactccctccatcccaaaaaatgtaattctaagtatgagttgtattattatttttggacaaaaggagtataccacaagaatgatatcatcgtcatgcttagatcctttttagtaaagcttgagcttctctaaaagtagagaaattagaaaaaaatcacgtttttgtggtcttgatttctagcctccacaaaatctttggttttacattttttgtttgattttggtttcagaagtccttatttatatgtgctagtttggcagcacttaaaatcgttagagagagcctaaacaaaagccttttcaaaacgaccttgagccagattggttgatggccaaaatttgattgtcaaaacttaggcaagccaagattttagcagctatttggtttggtaccaaaatttgccaatgatctgttcttttgccttttcaaccggtttatcagccgtacttcagcttattctctctcacagaacactattgaatcagccgaaaagccaccgcagaacaggaccagtatctcacaaatggcatgccaaatatactcaccgtcagtgagcccgtttaacggcgtcgacaagtctaacggccaccaaccagcgaaccaccagcgtcaagctagccaagcgaagcagacggccgagacgttgacaccttggcgcgggcatctctctggccccctctcgagagttccgctccacctccactggtggcggtttccaagtccgttccgcctcctgctcctcctcacacggcacgaaaccgtcacggcaccggcagcacgggggattcctttcccaccgctccttccctttcccttcctcgcccgccgttttaaatagccagccccatccccagcttctctccccaacctcagcttctctcgttgttcggagcgcacacacaacccgatccccaatcccctcgtctctcctcgcgagcctcgtcgatccccgcttcaaggtacggcgatcatcctccctttctctaccttctcttctctagactaggtcggcgatccatggttagggcctgctagttctgttcctgtttttccgtggctgcgaggtacaatagatctgatggcgttatgatggttaacttgtcatactcctgcggtgtgcggtctatagtgcttttaggacatcaatttgacctggctcgttcgagatcggcgatccatggttaggaccctaggcggtggagtcgggttagatccgcgctgtttgtgttagtagatggatgcgacctttacttcagacacgttctgattgttaacttgtcagcacctgggagtcctgggatggttctagctggttcgcagatgagatcgatttcatgatctgctgtatcttgtttcgttaggttccttttaatctatccgtggtattatgctaacctatgatatggttcgatcgtgctagctacgtcctgtgtcataatttttagcatgcccttttttgtttggttttgtctgattgggctgtagatcagagtatactgtttcaaactacctactggatatatttattaaatttgaatctgtatgtgtgtcacatatatcttcataattaaaatggatggaaagatatatggataggtacatgtgttgctgtgggttttactggtactttgttagatatacatgcttagatacatgaagcaacatgatgttacagttcaataattcttgtttacctaataaacaaataaggataggtgtatgttgctgtgggttttgctggtactttgttagatatatatgcttagatatatgaagcaacatcctgctacggtttaataattattgtttatatctaatagacaagcctgctttttaattattttgatatacttggatgatggcatacagcagctatgtgtggatttttaaatacccagcatcatgagcatgcatgaccctgccttagtatgctgtttatttgcttgagacttctttttttgttggtactcaccttttgtagtttggtgactcttctgcaggtgcaaccatgtctccggagaggagaccagttgagattaggccagctacagcagctgatatggccgcggtttgtgatatcgttaaccattacattgagacgtctacagtgaactttaggacagagccacaaacaccacaagagtggattgatgatctagagaggttgcaagatagatacccttggttggttgctgaggttgagggtgttgtggctggtattgcttacgctgggccctggaaggctaggaacgcttacgattggacagttgagagtactgtttacgtgtcacataggcatcaaaggttgggcctaggatccacattgtacacacatttgcttaagtctatggaggcgcaaggttttaagtctgtggttgctgttataggccttccaaacgatccatctgttaggttgcatgaggctttgggatacacagcccggggtacattgcgcgcagctggatacaagcatggtggatggcatgatgttggtttttggcaaagggattttgagttgccagctcctccaaggccagttaggccagttacccagatctgatacgcgctgctagtagccaagtacctacctcgagggcacactgtaggcagtgtgccatattacaggttcagattggccgggacaaagagtacactgcgattttactatcctcggtatgctggtactacaggttcacattcacatggttactacctggcctgtggtatgctggtactacaggtgttgctctgaatagctcaggcttgacccaagtaagagcagtgcaaattcccaatttccagaaaacaggaggacctccaaaggacttcaatgtaattcaaatttctttcagaggtccttttgcaaggggctggatgtaaagtacttttataataatccaagccattgtgcttctcaaaaaaaggaaaagaaaaaaatttgttgcggcccggccgtgacggccacgagcgaactcctgcaggagcagactcgcattatcgatggagctctaccaaactggccctaggcattaacctaccatggatcacatcgtaaaaaaaaaaccctaccatggatcctatctgttttctttttgccctgaaagagtgaagtcatcatcatatttaccatggcgcgcgtaggagcgcttcgtcgaagacccataggggggcggtactcgcaccgtggttgtttcctgttatgtaatatcggatgggggagcagtcggctaggttggtcccatcggtactggtcgtcccctagtgcgctagatgcgcgatgtttgtcctcaaaaactcttttcttcttaataacaatcatacgcaaattttttgcgtattcgagaaaaaaagaagattctatctgttttttttttgaaatggctccaatttataggaggagcccgtttaacggcgtcgacaaatctaacggacaccaaccagcgaatgagcgaacccaccagcgccaagctagccaagcgaagcagacggccgagacgctgacacccttgccttggcgcggcatctccgtcgctggctcgctggctctggccccttcgcgagagttccggtccacctccacctgtgtcggtttccaactccgttccgccttcgcgtgggacttgttccgttcatccgttggcggcatccggaaattgcgtggcgtagagcacggggccctcctctcacacggcacggaaccgtcacgagctcacggcaccggcagcacggcggggattccttccccaccaccgctccttccctttcccttcctcgcccgccatcataaatagccacccctcccagcttccttcgccacatcctctcatcatcttctctcgtgtagcacgcgcagcccgatccccaatcccctctcctcgcgagcctcgtcgatccctcgcttcaaggtatggctatcgtccttcctctctctctctttaccttatctagatcggcgatccatggttagggcctgctagttctccgttcgtgtttgtcgatggctgtgaggcacaatagatccgtcggcgttatgatggttagcctgtcatgctcttgcgatctgtggttcctttaggaaaggcattaatttaatccctgatggttcgagatcggtgatccatggttagtaccctaagctgtggagtcgggtttagatccgcgctgttcgtaggcgatctgttctgattgttaacttgtcagtacctgcgaatcctcggtggttctagctggttcggagatcagatcgattccattatctgctatacatcttgtttcgttgcctaggctccgtttaatctatccatcgtatgatgttagcctttgatatgattcgatcgtgctagctatgtcctgtggacttaattgtcaggtcctaatttttaggaagactgttccaaaccatctgctggatttattaaatttggatctggatgtgtcacatacaccttcataattaaaatggatggaaatatctcttatcttttagatatggataggcatttatatgatgctgtgagttttactagtactttcttagaatatatgtacttttttagacggaatattgatatgtatacatgtgtagatacatgaagcaacatgctgctgtagtctaataattcctgttcatctaataatcaagtatgtatatgttctgtgtgttttattggtatttgattagatatatacatgcttagatacatacatgaagcagcatgctgctacagtttaatcattattgtttatccaataaacaaacatgctttttaatttatcttgatatgcttggatgacggaatatgcagagattttaagtacccagcatcatgagcatgcatgaccctgcgttagtatgctgtttatttgcttgagactctttcttttgtagatactcaccctgttttctggtgatcctactgcaggtgaccggtcgccatggccaccgccaccactaccgccaccgctgcgttctccggcgtggtgagcgtcggcactgagacgcgcaggatctactccttcagccacctccagccttctgctgcgttccccgctaagccgtcttcgttcaagagcctgaagctgaaacagtccgcacgccttacccggcgcctggaccataggccattcgttgtcaggtgcatgctcaccttcgttaggaacgcctggtacgtcgccgctctccctgaggagctgagcgagaagcccttgggtcgcaccatcctagacactccgttagccctttaccgccagcctgacggcgtagtggcggccctgcttgacatctgcccgcataggttcgctccgctcagcgacggcatcctcgtcaacgggcatcttcagtgcccgtaccacgggctggaatttgacggcggtgggcagtgtgtccacaacccgcacggcaacggcgcacggccagcttccctcaacgttaggtcgttccctgttgtcgagcgcgacgcactgatctggatctggcctggcgacccagctctggccgatccaggagccattcccgacttcggttgccgcgtggacccagcctatcggacggtcggcggttacgggcacgtcgattgtaactataagctccttgtggacaaccttatggatttgggccacgctcagtacgtgcaccgggctaacgctcagactgacgcctttgaccgtctcgaaagggaggtcatcgtcggcgacggagagattcaggcgctgatgaagatccctggaggcacgccctctgtgctcatggcgaagtttctcagaggcgcgaacacgcccgtggacgcctggaacgacatccgctggaataaggtctccgcgatgctgaacttcatcgccgttgcgcccgagggcacacccaaagagcagtcaatccacagcagagggacccatattcttacaccggaaaccgaggctagttgccactacttcttcggctcgtcacggaatttcgggatagacgatccggagatggacggtgttcttcgatcttggcaagcgcaagctctcgtcaaggaagataaggtggtcgtggaggctatcgagcgtaggcgcgcctacgttgaggcgaacggtattaggcccgcgatgctgtcctgcgacgaggccgcagttagagtgtcgcgcgagatagaaaagctggagcagctagaggccgcctgattaattaaggccaaggcgatctatgactgaattgccaatgcaccagcctgtctacatgatgaataaataaagagtccatccagtgtgatggctcatgcctgtgtgagtgtgactgaatccatcagtgtgtgtgtgtgtttgtgtcaaccatgtgtgaatcaggtgtcaaaaatcgtggctggaaatccatgtggtttctagctttatgtaaatgttgtttgtgaaatataaatattgttttgtgtatgtgaattttactctctcatttttctcttgcactcaccattctattatagtaatttttttaagcggccgctgatgtatccgtccacggtggtgtgtccaatcagtgaataatctagttagtgaagccagaagtccatagtgccccttgctctgtcaccatatatccagttcaaccgcaccaatttgccatctcgaactggttcatgttttattcaggttggtaaatgaattttgccaattcaatgtagttagatatttccatgtcattttagtacatttaccaattttttatattctggctagaaaaggagaatggtgacgtctttcggaagatcaagatcaattatcaagtatcagcaacagcacctgaaggttggagtgcattagttgtcattgagaataatgctagctattcattgcactggcattagagacagagagggcgagccagtttgacatggcaaattagcacagtcaaactggatacgtggtgacggagggaggggcactatgaatttttggtgacggagggaggggcactatgaatttttggctttgctgacgggacacgccactatggatgaaattggacaaaatacgaatattcaaggatgaaagtggtcggtttgatagttcagggatgaaatgtgtctttgggcaaactttgaggacgaagttgcctattttgcattaaacgaatatatttatataccccaaaaaaaagaatacacatctccactccgagccggcatgtggggtccccactagtcagccactgtatggcgccgactagctcaacggccacgaaccagccaaccaccagcgcaacctaaacggcgtaaacgttgacggcatctctctctcgccccgtctcgaagcttccgcaccgctcgctggtcgctgcccggcgccgctcgtgctggactctttccgtggcggcttccgcgaaattgcgtggtggagaggagagacggaaccgtcacggcactggattccttccccacccggcttggccggcccctcctcgcctccataaataggcaccccgtcctcgcctcctctccccacctcatctcctcctttcccgtgaaccgtgaacacaacccgacccagatcccctcttgcgagcttcgtcgatccctcctccgcgtcaaggtacggagcttctcctcccccttcttctctagatcggcgtgttatgttgtttccgtggttgcttggttggatgaatcgaatgattcttagggcctaggaggctggttagatctgttgcgttctgtttcgtagatggattttggtgtaagatcaggtcggttccgctgtttaacttgtgatgctagtgtgatttttgggaggatttgagttgttaatctgggagttgttgggaggttctcgtaggcggattgtagatgaagtcgcccgcacgatttgcgtggcttgttgggtagctagggttagatctgctcggatttttcattgttacttattgagagataatgtagctaacctttacttgttcatctatgtatctcgtattcgtattcatctggttcgatggtgctagatagatgcgcctgatttgtccgatcgaattgggtagcatccgcggcttgtttggtagtgttctgattgatttgtcgctctagatctgagtggaataatattacatctcaacatgttactagaaacttggtttatagctccggatttacatgtttattcttatgtaaggttttaaatgaaagatttatgctactgctgctcgttgatcctttagcatccacctgaggaacatgcatgcatctgttacttcttttgatatatgcttagatagttgttagtatatactgctgttgttcgatgatccttcaggatgaacatgcatgatcatgttacttgtttttatatgcttctgctgttcgttgattctttagtactacctacctgatcatcttgcatgtttcctgcttgttagagattaattgattaggcttaccttgttgcctggtgattcttccttgcaggtgggtacccggaccgatggcaacagcaacatcagcttctctgttttcaactgtttcttcatcttactccaaagctagctccataccacattcaagactccaatctgtgaaattcaactcagtccctagcttcaccggtctcaaatcaacctctctcatctccggatctgattcctcttccttagccaagactctacgcggttccgtaacgaaagcacaaacatctgacaagaagccttacggattcaaaatcaacgctatgcacgcggcgctgactcctctcaccaacaagtatcgctttatcgacgtgcagccgctgacaggcgtcctcggtgcagagattacaggcgtggatctgcgggagcctctcgatgacagcacttggaatgagatcctggacgcctttcacacctaccaagtgatctactttccgggtcaagctatcactaacgagcagcacatcgcgttctcccgccggttcggccctgtggacccggtgccgatcttaaagagtatcgagggctatccagaggtgcagatgatacggcgcgaggcgaacgagagcagccggttcatcggagatgactggcacaccgattccaccttcctggacgctccgcctgccgccgtggtgatgagagctatcgaagtgccggagtatggaggtgacacaggcttcctctccatgtacagtgcctgggagacactctcgcctacgatgcaagctaccatcgaaggcttaaacgtggtccactcggcgacgaaggtcttcgggtcattgtaccaggcgactaattggcgcttctcgaacaccagcgtgaaagtgatggacgtggacgccggagatagagagactgtgcacccactcgtcgtgacgcatcctgttacgggaaggcgcgcactctactgcaaccaggtgtactgccagaagatccagggaatgacggacgcggagtcgaagtccctgttgcaattcctttacgagcacgccaccaagttcgacttcacctgccgggtccggtggaagaaggaccaagtcctggtgtgggacaacctgtgtaccatgcaccgcgccgtcccggactacgctgggaaattcagatacctgacccgcaccaccgtggcgggagacaagccgtcgcgttgacggtccgttaattaatcgagtgtgaaggaagtgaactgagtctcaagaataaaaactgcaagtatggcgctccattccatggaagacctgcatgcatcctatatatgtgcttttatgttcaagttggagaactatgtgtgttgtctttaagttggagtactctaagctattcgatctggagattatgctgtttttaataaaagtttgaagtgtatctgtcctgtttaattagtttcaagaaagccaagcgtgtttgggttctaggatgaacaaagtcgtccaagatgcaagaagttctagagaggtagctacatttctggaaattgttgcatcttcctttcttcaatatatatatattgtcctatttcataatgtcattctagccagctatctatattctatatatccatttccgttgccatactttattcactatgttgcatcgagtgagctgcattgctctgtactacatgttacttgatatgtgttgttcataaacacacacattaataatgatcagattgtgaaaaatacgcgtccgatcctacctgtcacttcatcaaaaggacagtagaaaaggaaggtggcacctacaaatgccatcattgcgataaaggaaaggctatcattcaagatgcctctgccgacagtggtcccaaagatggacccccacccacgaggagcatcgtggaaaaagaagacgttccaaccacgtcttcaaagcaagtggattgatgtgatacttccactgacgtaagggatgacgcacaatcccactatccttcgcaagacccttcctctatataaggaagttcatttcatttggagaggacacgctgaaatcaccagtctctctctacaagatcggggatctctagccctagaaccatcttccacacactcaagccacactattggagaacacacagggacaacacaccataagatccaagggaggcctccgccgccgccggtaaccaccccgcccctctcctctttctttctccgtttttttttccgtctcggtctcgatctttggccttggtagtttgggtgggcgagaggcggcttcgtgcgcgcccagatcggtgcgcgggaggggcgggatctcgcggctggggctctcgccggcgtggatccggcccggatctcgcggggaatggggctctcggatgtagatctgcgatccgccgttgttgggggagatgatggggggtttaaaatttccgccgtgctaaacaagatcaggaagaggggaaaagggcactatggtttatatttttatatatttctgctgcttcgtcaggcttagatgtgctagatctttctttcttctttttgtgggtagaatttgaatccctcagcattgttcatcggtagtttttcttttcatgatttgtgacaaatgcagcctcgtgcggagcttttttgtaggtagaagtgatcaaccatggcgcaagttagcagaatctgcaatggtgtgcagaacccatctcttatctccaatctctcgaaatccagtcaacgcaaatctcccttatcggtttctctgaagacgcagcagcatccacgagcttatccgatttcgtcgtcgtggggattgaagaagagtgggatgacgttaattggctctgagcttcgtcctcttaaggtcatgtcttctgtttccacggcgtgcatgcttcatggagcttcatctaggccagctactgccaggaagtctagcgggctcagtggcaccgtgcgcatccctggcgataaaagtatttcacacaggagcttcatgttcggaggacttgctagtggagagacgagaatcactggtttgcttgagggcgaagatgttatcaacaccggtaaggcgatgcaagcaatgggtgccagaatccgaaaagagggcgatacgtggatcatcgacggtgttggtaacggaggattgctcgctcccgaagcgccacttgactttgggaacgcagctacggggtgccgtcttactatgggactggtaggcgtgtatgactttgactctaccttcatcggtgacgcgagcctcactaagagaccaatgggacgagtgctgaatcccctgagggagatgggtgtccaggtgaaatctgaggatggtgatcgtcttccggttactctgcgaggccccaagacccccacgccaatcacgtacagggttccgatggcgtcagcacaggtcaagtcagcggtactcctggcgggcctcaacacacctggaatcacaaccgtgattgaacccatcatgactagagaccacacggagaagatgttgcagggtttcggcgctaatctaacggtcgaaaccgacgccgacggcgtgaggacaatccgcttggagggcagaggtaaactgactggccaagtcatcgatgtgcctggagatccctcgtccacagcgtttcccctcgtagctgcgttgctcgtccctggatctgatgtgacgatcctgaatgtcctcatgaatccaactagaaccggcctcatcctcacattgcaggagatgggtgctgacatcgaggttatcaatcctaggttggcaggtggagaggatgtggccgatctgcgcgtgcgttctagtacactcaaaggcgtgaccgtccctgaggatcgcgctccatccatgatcgacgagtaccccattctcgccgttgctgctgcgtttgccgagggcgcaactgtaatgaacggccttgaggagttgagggttaaggagagtgacaggctgtccgcggtggcgaatggcctgaagctaaacggcgtggactgcgacgaaggtgaaacgtcccttgtagtccgtggtcgcccagacgggaaggggttggggaatgcttcgggagctgctgtggcgacgcaccttgatcatagaatcgccatgtcatttctggtgatgggacttgtctccgagaatccggtgaccgttgacgatgctaccatgatcgccacctcctttcctgagttcatggacctcatggcaggcttgggggccaagatcgagctgtctgatactaaggccgcttgacacgtgagacgacgaccgtgcatggtgatgaatcacagacgacgaacacgcatgtcgcatcgccgtcctctttgtatcacacagcatcaccttcttcgctctactactcccccgagcaatcaccgaccaataacaccaaccatcaacctcccccgtcgccgccgccttcaccgtcctcccctcacaccatagaactgcaaatgtccgcctgcagggtggggcccatcgtggccagttatccttagctatccgtgtcagaatcatcttatcatcgagtcgagtcgttatcgtgtccagtggctctctcgagtcgagaagccctctatccatccatccagtgttaggtgttcttcgtccgtgatgttaccatgaattgagttcgctttggttatggtgtttgaactgcttgttgctatctatcggaatgaaatgaaatagaagacaaggagaaaaaaaagagttcgaaagttttgttcgcataccatatatttccttccggtgcgcgctgtttattcctcgctcagcagcaagattgtttgatcgatattgcagcaagcaattacacaataaatatattgctacactggtacttcaaactacactggtggtcggtgattttcaatagcatgaaccttaattgaacatctgtgtagcttacatctccttcgaaagctgcaatgcttgagaacttggaaagaaattcttgtgatggcagaagctattcactgtccttcgctgcatttacagtccatacagacacagcatttccattttgcacaagatagagaacaacaatcagccttttaggtcaatcccaagtgtgcatgacgtcccgcgatcgcccgcacaacaaacgcaccggtgcacaaactat

SEQ ID NO: 10 - DNA, 16068 bp, Artificial Sequence
  Chimeric DNA molecule of maize genomic DNA and transgene DNA
atctacagggcgcgcagcggctgacacatgggacccacgggcaaaggcagcggcagactcgcgcgcgagagcacgcaagcaccgattgacgcgcgtgccccttttgtcggagaacgagggtgcgcgatcgtccgtgcatggttgagacggccaggcggggcccacccattggcgccatgccgcgcgagcagcagctggcccgcacaggtgcaaaggttgagtgggctagaagcgaagacctagtccaagcgacggtttcttccttttttctctttttttctttttcctttatattttcttgttttattttattttcatttttttattttcaaatctaaatttgaactcaagtgtgagattcatactttgaattaaatgctcacattcaaatatcagtaggaatagaatatttttaactatatgtttattttctctattttatacaatcttttccttttttcatttttaaacctcaatttgtaaattatatctaaattccaattttggtcattagtatactcctactaatatcattttattgttatgaaatgcacacacaataaactccaacttgatgaatagatatctatttattctaattaatttatttgtttggtagatgttcaaaatatgaaacacacacatattgttttctttctttttagaaaaatggtatttttattgtgggacaagaactaaaagtcacctcaaaattaaatactcatgtataatttgggatatctgaatttactatttttatttcttcatatatttaatttattattaattttttttcttattgggccttacacttatgagatcatagaggcatgtggatcagtggcatacaagttgaaattactgccaaaaatgtctgtcatacacaatccgtgtgtttggtttgtggaccagcagagcctggctactctaatccgtatgtagagaaccaagctcccacgagacagactcaatgtatccgagatactcttgtttggttacacttgcaaaaatagaccactcttgtttggtttcatgtccgggaaatctacatggatcagcaatgagtatgatggtcaatatggagaaaaagaaagagtaattaccaattttttttcaattcaaaaatgtagatgtccgcagcgttattataaaatgaaagtacattttgataaaacgacaaattacgatccgtcgtatttataggcgaaagcaataaacaaattattctaattcggaaatctttatttcgacgtgtctacattcacgtccaaatgggggcttagatgagaaacttcacgatttggcgcgactaactaagcactagcgtacgggacccagatatcgaattcaagctgaccgccaccggcaaacaaccacgaatttgtaatggtactaggcaaattctccgtttggcggtgtgtgccggccaattacacgtttttgcggtgtcctccgacaaaatttgccttttaaaaacaattttataagagaagctccggagataaaaggccgtcaatgttacaagagtgaagtcgtctactccctccatcccaaaaaatgtaattctaagtatgagttgtattattatttttggacaaaaggagtataccacaagaatgatatcatcgtcatgcttagatcctttttagtaaagcttgagcttctctaaaagtagagaaattagaaaaaaatcacgtttttgtggtcttgatttctagcctccacaaaatctttggttttacattttttgtttgattttggtttcagaagtccttatttatatgtgctagtttggcagcacttaaaatcgttagagagagcctaaacaaaagccttttcaaaacgaccttgagccagattggttgatggccaaaatttgattgtcaaaacttaggcaagccaagattttagcagctatttggtttggtaccaaaatttgccaatgatctgttcttttgccttttcaaccggtttatcagccgtacttcagcttattctctctcacagaacactattgaatcagccgaaaagccaccgcagaacaggaccagtatctcacaaatggcatgccaaatatactcaccgtcagtgagcccgtttaacggcgtcgacaagtctaacggccaccaaccagcgaaccaccagcgtcaagctagccaagcgaagcagacggccgagacgttgacaccttggcgcgggcatctctctggccccctctcgagagttccgctccacctccactggtggcggtttccaagtccgttccgcctcctgctcctcctcacacggcacgaaaccgtcacggcaccggcagcacgggggattcctttcccaccgctccttccctttcccttcctcgcccgccgttttaaatagccagccccatccccagcttctctccccaacctcagcttctctcgttgttcggagcgcacacacaacccgatccccaatcccctcgtctctcctcgcgagcctcgtcgatccccgcttcaaggtacggcgatcatcctccctttctctaccttctcttctctagactaggtcggcgatccatggttagggcctgctagttctgttcctgtttttccgtggctgcgaggtacaatagatctgatggcgttatgatggttaacttgtcatactcctgcggtgtgcggtctatagtgcttttaggacatcaatttgacctggctcgttcgagatcggcgatccatggttaggaccctaggcggtggagtcgggttagatccgcgctgtttgtgttagtagatggatgcgacctttacttcagacacgttctgattgttaacttgtcagcacctgggagtcctgggatggttctagctggttcgcagatgagatcgatttcatgatctgctgtatcttgtttcgttaggttccttttaatctatccgtggtattatgctaacctatgatatggttcgatcgtgctagctacgtcctgtgtcataatttttagcatgcccttttttgtttggttttgtctgattgggctgtagatcagagtatactgtttcaaactacctactggatatatttattaaatttgaatctgtatgtgtgtcacatatatcttcataattaaaatggatggaaagatatatggataggtacatgtgttgctgtgggttttactggtactttgttagatatacatgcttagatacatgaagcaacatgatgttacagttcaataattcttgtttacctaataaacaaataaggataggtgtatgttgctgtgggttttgctggtactttgttagatatatatgcttagatatatgaagcaacatcctgctacggtttaataattattgtttatatctaatagacaagcctgctttttaattattttgatatacttggatgatggcatacagcagctatgtgtggatttttaaatacccagcatcatgagcatgcatgaccctgccttagtatgctgtttatttgcttgagacttctttttttgttggtactcaccttttgtagtttggtgactcttctgcaggtgcaaccatgtctccggagaggagaccagttgagattaggccagctacagcagctgatatggccgcggtttgtgatatcgttaaccattacattgagacgtctacagtgaactttaggacagagccacaaacaccacaagagtggattgatgatctagagaggttgcaagatagatacccttggttggttgctgaggttgagggtgttgtggctggtattgcttacgctgggccctggaaggctaggaacgcttacgattggacagttgagagtactgtttacgtgtcacataggcatcaaaggttgggcctaggatccacattgtacacacatttgcttaagtctatggaggcgcaaggttttaagtctgtggttgctgttataggccttccaaacgatccatctgttaggttgcatgaggctttgggatacacagcccggggtacattgcgcgcagctggatacaagcatggtggatggcatgatgttggtttttggcaaagggattttgagttgccagctcctccaaggccagttaggccagttacccagatctgatacgcgctgctagtagccaagtacctacctcgagggcacactgtaggcagtgtgccatattacaggttcagattggccgggacaaagagtacactgcgattttactatcctcggtatgctggtactacaggttcacattcacatggttactacctggcctgtggtatgctggtactacaggtgttgctctgaatagctcaggcttgacccaagtaagagcagtgcaaattcccaatttccagaaaacaggaggacctccaaaggacttcaatgtaattcaaatttctttcagaggtccttttgcaaggggctggatgtaaagtacttttataataatccaagccattgtgcttctcaaaaaaaggaaaagaaaaaaatttgttgcggcccggccgtgacggccacgagcgaactcctgcaggagcagactcgcattatcgatggagctctaccaaactggccctaggcattaacctaccatggatcacatcgtaaaaaaaaaaccctaccatggatcctatctgttttctttttgccctgaaagagtgaagtcatcatcatatttaccatggcgcgcgtaggagcgcttcgtcgaagacccataggggggcggtactcgcaccgtggttgtttcctgttatgtaatatcggatgggggagcagtcggctaggttggtcccatcggtactggtcgtcccctagtgcgctagatgcgcgatgtttgtcctcaaaaactcttttcttcttaataacaatcatacgcaaattttttgcgtattcgagaaaaaaagaagattctatctgttttttttttgaaatggctccaatttataggaggagcccgtttaacggcgtcgacaaatctaacggacaccaaccagcgaatgagcgaacccaccagcgccaagctagccaagcgaagcagacggccgagacgctgacacccttgccttggcgcggcatctccgtcgctggctcgctggctctggccccttcgcgagagttccggtccacctccacctgtgtcggtttccaactccgttccgccttcgcgtgggacttgttccgttcatccgttggcggcatccggaaattgcgtggcgtagagcacggggccctcctctcacacggcacggaaccgtcacgagctcacggcaccggcagcacggcggggattccttccccaccaccgctccttccctttcccttcctcgcccgccatcataaatagccacccctcccagcttccttcgccacatcctctcatcatcttctctcgtgtagcacgcgcagcccgatccccaatcccctctcctcgcgagcctcgtcgatccctcgcttcaaggtatggctatcgtccttcctctctctctctttaccttatctagatcggcgatccatggttagggcctgctagttctccgttcgtgtttgtcgatggctgtgaggcacaatagatccgtcggcgttatgatggttagcctgtcatgctcttgcgatctgtggttcctttaggaaaggcattaatttaatccctgatggttcgagatcggtgatccatggttagtaccctaagctgtggagtcgggtttagatccgcgctgttcgtaggcgatctgttctgattgttaacttgtcagtacctgcgaatcctcggtggttctagctggttcggagatcagatcgattccattatctgctatacatcttgtttcgttgcctaggctccgtttaatctatccatcgtatgatgttagcctttgatatgattcgatcgtgctagctatgtcctgtggacttaattgtcaggtcctaatttttaggaagactgttccaaaccatctgctggatttattaaatttggatctggatgtgtcacatacaccttcataattaaaatggatggaaatatctcttatcttttagatatggataggcatttatatgatgctgtgagttttactagtactttcttagaatatatgtacttttttagacggaatattgatatgtatacatgtgtagatacatgaagcaacatgctgctgtagtctaataattcctgttcatctaataatcaagtatgtatatgttctgtgtgttttattggtatttgattagatatatacatgcttagatacatacatgaagcagcatgctgctacagtttaatcattattgtttatccaataaacaaacatgctttttaatttatcttgatatgcttggatgacggaatatgcagagattttaagtacccagcatcatgagcatgcatgaccctgcgttagtatgctgtttatttgcttgagactctttcttttgtagatactcaccctgttttctggtgatcctactgcaggtgaccggtcgccatggccaccgccaccactaccgccaccgctgcgttctccggcgtggtgagcgtcggcactgagacgcgcaggatctactccttcagccacctccagccttctgctgcgttccccgctaagccgtcttcgttcaagagcctgaagctgaaacagtccgcacgccttacccggcgcctggaccataggccattcgttgtcaggtgcatgctcaccttcgttaggaacgcctggtacgtcgccgctctccctgaggagctgagcgagaagcccttgggtcgcaccatcctagacactccgttagccctttaccgccagcctgacggcgtagtggcggccctgcttgacatctgcccgcataggttcgctccgctcagcgacggcatcctcgtcaacgggcatcttcagtgcccgtaccacgggctggaatttgacggcggtgggcagtgtgtccacaacccgcacggcaacggcgcacggccagcttccctcaacgttaggtcgttccctgttgtcgagcgcgacgcactgatctggatctggcctggcgacccagctctggccgatccaggagccattcccgacttcggttgccgcgtggacccagcctatcggacggtcggcggttacgggcacgtcgattgtaactataagctccttgtggacaaccttatggatttgggccacgctcagtacgtgcaccgggctaacgctcagactgacgcctttgaccgtctcgaaagggaggtcatcgtcggcgacggagagattcaggcgctgatgaagatccctggaggcacgccctctgtgctcatggcgaagtttctcagaggcgcgaacacgcccgtggacgcctggaacgacatccgctggaataaggtctccgcgatgctgaacttcatcgccgttgcgcccgagggcacacccaaagagcagtcaatccacagcagagggacccatattcttacaccggaaaccgaggctagttgccactacttcttcggctcgtcacggaatttcgggatagacgatccggagatggacggtgttcttcgatcttggcaagcgcaagctctcgtcaaggaagataaggtggtcgtggaggctatcgagcgtaggcgcgcctacgttgaggcgaacggtattaggcccgcgatgctgtcctgcgacgaggccgcagttagagtgtcgcgcgagatagaaaagctggagcagctagaggccgcctgattaattaaggccaaggcgatctatgactgaattgccaatgcaccagcctgtctacatgatgaataaataaagagtccatccagtgtgatggctcatgcctgtgtgagtgtgactgaatccatcagtgtgtgtgtgtgtttgtgtcaaccatgtgtgaatcaggtgtcaaaaatcgtggctggaaatccatgtggtttctagctttatgtaaatgttgtttgtgaaatataaatattgttttgtgtatgtgaattttactctctcatttttctcttgcactcaccattctattatagtaatttttttaagcggccgctgatgtatccgtccacggtggtgtgtccaatcagtgaataatctagttagtgaagccagaagtccatagtgccccttgctctgtcaccatatatccagttcaaccgcaccaatttgccatctcgaactggttcatgttttattcaggttggtaaatgaattttgccaattcaatgtagttagatatttccatgtcattttagtacatttaccaattttttatattctggctagaaaaggagaatggtgacgtctttcggaagatcaagatcaattatcaagtatcagcaacagcacctgaaggttggagtgcattagttgtcattgagaataatgctagctattcattgcactggcattagagacagagagggcgagccagtttgacatggcaaattagcacagtcaaactggatacgtggtgacggagggaggggcactatgaatttttggtgacggagggaggggcactatgaatttttggctttgctgacgggacacgccactatggatgaaattggacaaaatacgaatattcaaggatgaaagtggtcggtttgatagttcagggatgaaatgtgtctttgggcaaactttgaggacgaagttgcctattttgcattaaacgaatatatttatataccccaaaaaaaagaatacacatctccactccgagccggcatgtggggtccccactagtcagccactgtatggcgccgactagctcaacggccacgaaccagccaaccaccagcgcaacctaaacggcgtaaacgttgacggcatctctctctcgccccgtctcgaagcttccgcaccgctcgctggtcgctgcccggcgccgctcgtgctggactctttccgtggcggcttccgcgaaattgcgtggtggagaggagagacggaaccgtcacggcactggattccttccccacccggcttggccggcccctcctcgcctccataaataggcaccccgtcctcgcctcctctccccacctcatctcctcctttcccgtgaaccgtgaacacaacccgacccagatcccctcttgcgagcttcgtcgatccctcctccgcgtcaaggtacggagcttctcctcccccttcttctctagatcggcgtgttatgttgtttccgtggttgcttggttggatgaatcgaatgattcttagggcctaggaggctggttagatctgttgcgttctgtttcgtagatggattttggtgtaagatcaggtcggttccgctgtttaacttgtgatgctagtgtgatttttgggaggatttgagttgttaatctgggagttgttgggaggttctcgtaggcggattgtagatgaagtcgcccgcacgatttgcgtggcttgttgggtagctagggttagatctgctcggatttttcattgttacttattgagagataatgtagctaacctttacttgttcatctatgtatctcgtattcgtattcatctggttcgatggtgctagatagatgcgcctgatttgtccgatcgaattgggtagcatccgcggcttgtttggtagtgttctgattgatttgtcgctctagatctgagtggaataatattacatctcaacatgttactagaaacttggtttatagctccggatttacatgtttattcttatgtaaggttttaaatgaaagatttatgctactgctgctcgttgatcctttagcatccacctgaggaacatgcatgcatctgttacttcttttgatatatgcttagatagttgttagtatatactgctgttgttcgatgatccttcaggatgaacatgcatgatcatgttacttgtttttatatgcttctgctgttcgttgattctttagtactacctacctgatcatcttgcatgtttcctgcttgttagagattaattgattaggcttaccttgttgcctggtgattcttccttgcaggtgggtacccggaccgatggcaacagcaacatcagcttctctgttttcaactgtttcttcatcttactccaaagctagctccataccacattcaagactccaatctgtgaaattcaactcagtccctagcttcaccggtctcaaatcaacctctctcatctccggatctgattcctcttccttagccaagactctacgcggttccgtaacgaaagcacaaacatctgacaagaagccttacggattcaaaatcaacgctatgcacgcggcgctgactcctctcaccaacaagtatcgctttatcgacgtgcagccgctgacaggcgtcctcggtgcagagattacaggcgtggatctgcgggagcctctcgatgacagcacttggaatgagatcctggacgcctttcacacctaccaagtgatctactttccgggtcaagctatcactaacgagcagcacatcgcgttctcccgccggttcggccctgtggacccggtgccgatcttaaagagtatcgagggctatccagaggtgcagatgatacggcgcgaggcgaacgagagcagccggttcatcggagatgactggcacaccgattccaccttcctggacgctccgcctgccgccgtggtgatgagagctatcgaagtgccggagtatggaggtgacacaggcttcctctccatgtacagtgcctgggagacactctcgcctacgatgcaagctaccatcgaaggcttaaacgtggtccactcggcgacgaaggtcttcgggtcattgtaccaggcgactaattggcgcttctcgaacaccagcgtgaaagtgatggacgtggacgccggagatagagagactgtgcacccactcgtcgtgacgcatcctgttacgggaaggcgcgcactctactgcaaccaggtgtactgccagaagatccagggaatgacggacgcggagtcgaagtccctgttgcaattcctttacgagcacgccaccaagttcgacttcacctgccgggtccggtggaagaaggaccaagtcctggtgtgggacaacctgtgtaccatgcaccgcgccgtcccggactacgctgggaaattcagatacctgacccgcaccaccgtggcgggagacaagccgtcgcgttgacggtccgttaattaatcgagtgtgaaggaagtgaactgagtctcaagaataaaaactgcaagtatggcgctccattccatggaagacctgcatgcatcctatatatgtgcttttatgttcaagttggagaactatgtgtgttgtctttaagttggagtactctaagctattcgatctggagattatgctgtttttaataaaagtttgaagtgtatctgtcctgtttaattagtttcaagaaagccaagcgtgtttgggttctaggatgaacaaagtcgtccaagatgcaagaagttctagagaggtagctacatttctggaaattgttgcatcttcctttcttcaatatatatatattgtcctatttcataatgtcattctagccagctatctatattctatatatccatttccgttgccatactttattcactatgttgcatcgagtgagctgcattgctctgtactacatgttacttgatatgtgttgttcataaacacacacattaataatgatcagattgtgaaaaatacgcgtccgatcctacctgtcacttcatcaaaaggacagtagaaaaggaaggtggcacctacaaatgccatcattgcgataaaggaaaggctatcattcaagatgcctctgccgacagtggtcccaaagatggacccccacccacgaggagcatcgtggaaaaagaagacgttccaaccacgtcttcaaagcaagtggattgatgtgatacttccactgacgtaagggatgacgcacaatcccactatccttcgcaagacccttcctctatataaggaagttcatttcatttggagaggacacgctgaaatcaccagtctctctctacaagatcggggatctctagccctagaaccatcttccacacactcaagccacactattggagaacacacagggacaacacaccataagatccaagggaggcctccgccgccgccggtaaccaccccgcccctctcctctttctttctccgtttttttttccgtctcggtctcgatctttggccttggtagtttgggtgggcgagaggcggcttcgtgcgcgcccagatcggtgcgcgggaggggcgggatctcgcggctggggctctcgccggcgtggatccggcccggatctcgcggggaatggggctctcggatgtagatctgcgatccgccgttgttgggggagatgatggggggtttaaaatttccgccgtgctaaacaagatcaggaagaggggaaaagggcactatggtttatatttttatatatttctgctgcttcgtcaggcttagatgtgctagatctttctttcttctttttgtgggtagaatttgaatccctcagcattgttcatcggtagtttttcttttcatgatttgtgacaaatgcagcctcgtgcggagcttttttgtaggtagaagtgatcaaccatggcgcaagttagcagaatctgcaatggtgtgcagaacccatctcttatctccaatctctcgaaatccagtcaacgcaaatctcccttatcggtttctctgaagacgcagcagcatccacgagcttatccgatttcgtcgtcgtggggattgaagaagagtgggatgacgttaattggctctgagcttcgtcctcttaaggtcatgtcttctgtttccacggcgtgcatgcttcatggagcttcatctaggccagctactgccaggaagtctagcgggctcagtggcaccgtgcgcatccctggcgataaaagtatttcacacaggagcttcatgttcggaggacttgctagtggagagacgagaatcactggtttgcttgagggcgaagatgttatcaacaccggtaaggcgatgcaagcaatgggtgccagaatccgaaaagagggcgatacgtggatcatcgacggtgttggtaacggaggattgctcgctcccgaagcgccacttgactttgggaacgcagctacggggtgccgtcttactatgggactggtaggcgtgtatgactttgactctaccttcatcggtgacgcgagcctcactaagagaccaatgggacgagtgctgaatcccctgagggagatgggtgtccaggtgaaatctgaggatggtgatcgtcttccggttactctgcgaggccccaagacccccacgccaatcacgtacagggttccgatggcgtcagcacaggtcaagtcagcggtactcctggcgggcctcaacacacctggaatcacaaccgtgattgaacccatcatgactagagaccacacggagaagatgttgcagggtttcggcgctaatctaacggtcgaaaccgacgccgacggcgtgaggacaatccgcttggagggcagaggtaaactgactggccaagtcatcgatgtgcctggagatccctcgtccacagcgtttcccctcgtagctgcgttgctcgtccctggatctgatgtgacgatcctgaatgtcctcatgaatccaactagaaccggcctcatcctcacattgcaggagatgggtgctgacatcgaggttatcaatcctaggttggcaggtggagaggatgtggccgatctgcgcgtgcgttctagtacactcaaaggcgtgaccgtccctgaggatcgcgctccatccatgatcgacgagtaccccattctcgccgttgctgctgcgtttgccgagggcgcaactgtaatgaacggccttgaggagttgagggttaaggagagtgacaggctgtccgcggtggcgaatggcctgaagctaaacggcgtggactgcgacgaaggtgaaacgtcccttgtagtccgtggtcgcccagacgggaaggggttggggaatgcttcgggagctgctgtggcgacgcaccttgatcatagaatcgccatgtcatttctggtgatgggacttgtctccgagaatccggtgaccgttgacgatgctaccatgatcgccacctcctttcctgagttcatggacctcatggcaggcttgggggccaagatcgagctgtctgatactaaggccgcttgacacgtgagacgacgaccgtgcatggtgatgaatcacagacgacgaacacgcatgtcgcatcgccgtcctctttgtatcacacagcatcaccttcttcgctctactactcccccgagcaatcaccgaccaataacaccaaccatcaacctcccccgtcgccgccgccttcaccgtcctcccctcacaccatagaactgcaaatgtccgcctgcagggtggggcccatcgtggccagttatccttagctatccgtgtcagaatcatcttatcatcgagtcgagtcgttatcgtgtccagtggctctctcgagtcgagaagccctctatccatccatccagtgttaggtgttcttcgtccgtgatgttaccatgaattgagttcgctttggttatggtgtttgaactgcttgttgctatctatcggaatgaaatgaaatagaagacaaggagaaaaaaaagagttcgaaagttttgttcgcataccatatatttccttccggtgcgcgctgtttattcctcgctcagcagcaagattgtttgatcgatattgcagcaagcaattacacaataaatatattgctacactggtacttcaaactacactggtggtcggtgattttcaatagcatgaaccttaattgaacatctgtgtagcttacatctccttcgaaagctgcaatgcttgagaacttggaaagaaattcttgtgatggcagaagctattcactgtccttcgctgcatttacagtccatacagacacagcatttccattttgcacaagatagagaacaacaatcagccttttaggtcaatcccaagtgtgcatgacgtcccgcgatcgcccgcacaacaaacgcaccggtgcacaaactatagcaagtgtggtctatttttatatagcaagtgaggtcagataaaataataaataaaatcattaaattttatatagcaagtgtggtctatttttgcttgtaaactacagagaatatatatatgttaaatcggtagaacaattggctatttaaactaaaagatttaaaaaaaacaaagataaaaaatgtttttgaactgcgtgtctcgagagcagccagcatgcttccgacctgcatgagcagcgatgctcctggtgaccgcacgaacggaacctggcccgatggatgattttgcatcaacagcgcctgtatgcaacgatcatccaaccaaacatacttcgctttgaggatccacgcctacaacgtccgcgctcgtccatgcaaccaaacacacggaatgtgttccatgtgtcccaattgaaagaagtgtattcggttaacaacggaagtcataaccgagccagatatagagatagaaccagatctatcataccaagaacacccctccaagattctagactgcaaggaaagatccactcgtgcgaagacgaccaagatgtataagatccaatggagcaaccatacggaagaagaggctacgtgggagactgaggattatctatgcaaatactaccccgattgtctacctaaggaagtcagtacgtaaccatgccccagccccctgccctccgattccaaatatagaaaagatactcttaatgaaaactgaattaagaaatgaaattaagcgaagaaggacttccttctgaagttgcaaagaggatggcattcgaagagcagatttttctcgcgaaccttaaaaagctaaccaatactatgcaagcaagctataaccacctcctcactcctgggtgatctcgactcgaatctcggggcgagattcttttaaggggggagagctgtaacaccccaggtgttacttagggtttcccccttagtacctccatttgtgacctattatcacatgtggtttggtttaagaaaaaggcaccaaacttgaggggccaagccc

SEQ ID NO: 11 - DNA, 29 bp, Artificial Sequence
  Chemically Synthesized Oligonucleotide PCR Primer
ttgctatataaaaatagaccacacttgct

SEQ ID NO: 12 - DNA, 17 bp, Artificial Sequence
  Chemically Synthesized Oligonucleotide PCR Primer
catgacgtcccgcgatc

SEQ ID NO: 13 - DNA, 16 bp, Artificial Sequence
  Chemically Synthesized Oligonucleotide PCR Probe
cacaacaaacgcaccg